European Patent Application EP 4 219 710 A2, published August 2, 2023. Title: TAGGING NUCLEIC ACIDS FOR SEQUENCE ASSEMBLY. Applicant: DOVETAIL GENOMICS LLC. Application EP. The sequence listing filed with the application follows.

SEQUENCE LISTING (34 sequences)

SEQ ID NO: 1 - DNA, 33 bp, synthetic construct
  misc_feature 1..33: note = Description of Artificial Sequence: Synthetic oligonucleotide
  source 1..33: mol_type = other DNA
acactctttccctacacgacgctcttccgatct

SEQ ID NO: 2 - DNA, 31 bp, synthetic construct
  misc_feature 1..31: note = Description of Artificial Sequence: Synthetic oligonucleotide
  source 1..31: mol_type = other DNA
aaaaagatatcacgtacgtacgtacgtacgt

SEQ ID NO: 3 - DNA, 84 bp, synthetic construct
  misc_feature 1..84: note = Description of Artificial Sequence: Synthetic oligonucleotide
  misc_difference 32..51
  source 1..84: mol_type = other DNA
aaaaagatatcacgtacgtacgtacgtacgtnnnnnnnnnnnnnnnnnnnnagatcggaagagcgtcgtgtagggaaagagtgt

SEQ ID NO: 4 - DNA, 84 bp, synthetic construct
  misc_feature 1..84: note = Description of Artificial Sequence: Synthetic oligonucleotide
  misc_difference 34..53
  source 1..84: mol_type = other DNA
acactctttccctacacgacgctcttccgatctnnnnnnnnnnnnnnnnnnnnacgtacgtacgtacgtacgtgatatcttttt

SEQ ID NO: 5 - DNA, 76 bp, synthetic construct
  misc_feature 1..76: note = Description of Artificial Sequence: Synthetic oligonucleotide
  misc_difference 34..53
  source 1..76: mol_type = other DNA
acactctttccctacacgacgctcttccgatctnnnnnnnnnnnnnnnnnnnnacgtacgtacgtacgtacgtgat

SEQ ID NO: 6 - DNA, 29 bp, synthetic construct
  misc_feature 1..29: note = Description of Artificial Sequence: Synthetic oligonucleotide
  misc_difference 1..6
  source 1..29: mol_type = other DNA
nnnnnnatcacgtacgtacgtacgtacgt

SEQ ID NO: 7 - DNA, 82 bp, synthetic construct
  misc_feature 1..82: note = Description of Artificial Sequence: Synthetic oligonucleotide
  misc_difference 34..53
  misc_difference 77..82
  source 1..82: mol_type = other DNA
acactctttccctacacgacgctcttccgatctnnnnnnnnnnnnnnnnnnnnacgtacgtacgtacgtacgtgatnnnnnn

SEQ ID NO: 8 - DNA, 82 bp, synthetic construct
  misc_feature 1..82: note = Description of Artificial Sequence: Synthetic oligonucleotide
  misc_difference 1..6
  misc_difference 30..49
  source 1..82: mol_type = other DNA
nnnnnnatcacgtacgtacgtacgtacgtnnnnnnnnnnnnnnnnnnnnagatcggaagagcgtcgtgtagggaaagagtgt

SEQ ID NO: 9 - DNA, 83 bp, synthetic construct
  misc_feature 1..83: note = Description of Artificial Sequence: Synthetic oligonucleotide
  misc_difference 34..53
  misc_difference 77..82
  source 1..83: mol_type = other DNA
acactctttccctacacgacgctcttccgatctnnnnnnnnnnnnnnnnnnnnacgtacgtacgtacgtacgtgatnnnnnna

SEQ ID NO: 10 - DNA, 34 bp, synthetic construct
  misc_feature 1..34: note = Description of Artificial Sequence: Synthetic oligonucleotide
  source 1..34: mol_type = other DNA
agatcggaagagcacacgtctgaactccagtcac

SEQ ID NO: 11 - DNA, 35 bp, synthetic construct
  misc_feature 1..35: note = Description of Artificial Sequence: Synthetic oligonucleotide
  source 1..35: mol_type = other DNA
gtgactggagttcagacgtgtgctcttccgatctt

SEQ ID NO: 12 - DNA, 117 bp, synthetic construct
  misc_feature 1..117: note = Description of Artificial Sequence: Synthetic polynucleotide
  misc_difference 34..53
  misc_difference 77..82
  source 1..117: mol_type = other DNA
acactctttccctacacgacgctcttccgatctnnnnnnnnnnnnnnnnnnnnacgtacgtacgtacgtacgtgatnnnnnnaagatcggaagagcacacgtctgaactccagtcac

SEQ ID NO: 13 - DNA, 117 bp, synthetic construct
  misc_feature 1..117: note = Description of Artificial Sequence: Synthetic polynucleotide
  misc_difference 36..41
  misc_difference 65..84
  source 1..117: mol_type = other DNA
gtgactggagttcagacgtgtgctcttccgatcttnnnnnnatcacgtacgtacgtacgtacgtnnnnnnnnnnnnnnnnnnnnagatcggaagagcgtcgtgtagggaaagagtgt

SEQ ID NO: 14 - DNA, 20 bp, synthetic construct
  misc_feature 1..20: note = Description of Artificial Sequence: Synthetic oligonucleotide
  source 1..20: mol_type = other DNA
tcaagtggcagaagcacaag

SEQ ID NO: 15-16 - skipped (2 entries)

SEQ ID NO: 17 - DNA, 20 bp, synthetic construct
  misc_feature 1..20: note = Description of Artificial Sequence: Synthetic oligonucleotide
  source 1..20: mol_type = other DNA
tgcctttatggagtcgaacc

SEQ ID NO: 18 - DNA, 93 bp, synthetic construct
  misc_feature 1..93: note = Description of Artificial Sequence: Synthetic oligonucleotide
  misc_difference 25..40
  source 1..93: mol_type = other DNA
tgcctttatggagtcgaaccgatcnnnnnnnnnnnnnnnnagatcggaagagcgtcgtgtagggaaagagtgtcttgtgcttctgccacttga

SEQ ID NO: 19 - DNA, 20 bp, synthetic construct
  misc_feature 1..20: note = Description of Artificial Sequence: Synthetic oligonucleotide
  source 1..20: mol_type = other DNA
cttgtgcttctgccacttga

SEQ ID NO: 20 - DNA, 24 bp, synthetic construct
  misc_feature 1..24: note = Description of Artificial Sequence: Synthetic oligonucleotide
  source 1..24: mol_type = other DNA
tgcctttatggagtcgaaccgatc

SEQ ID NO: 21 - DNA, 24 bp, synthetic construct
  misc_feature 1..24: note = Description of Artificial Sequence: Synthetic oligonucleotide
  source 1..24: mol_type = other DNA
gatcggttcgactccataaaggca

SEQ ID NO: 22-24 - skipped (3 entries)

SEQ ID NO: 25 - DNA, 25 bp, synthetic construct
  misc_feature 1..25: note = Description of Artificial Sequence: Synthetic oligonucleotide
  misc_difference 13..24
  source 1..25: mol_type = other DNA
atgcatgcactannnnnnnnnnnnt

SEQ ID NO: 26 - DNA, 39 bp, synthetic construct
  misc_feature 1..39: note = Description of Artificial Sequence: Synthetic oligonucleotide
  misc_difference 13..24
  misc_difference 30..39
  source 1..39: mol_type = other DNA
atgcatgcactannnnnnnnnnnntgatcnnnnnnnnnn

SEQ ID NO: 27-28 - skipped (2 entries)

SEQ ID NO: 29 - DNA, 18 bp, synthetic construct
  misc_feature 1..18: note = Description of Artificial Sequence: Synthetic oligonucleotide
  misc_difference 1..7
  source 1..18: mol_type = other DNA
nnnnnnntcttcaagctt

SEQ ID NO: 30 - DNA, 11 bp, synthetic construct
  misc_feature 1..11: note = Description of Artificial Sequence: Synthetic oligonucleotide
  source 1..11: mol_type = other DNA
aagcttgaaga

SEQ ID NO: 31 - skipped

SEQ ID NO: 32 - DNA, 10 bp, synthetic construct
  misc_feature 1..10: note = Description of Artificial Sequence: Synthetic oligonucleotide
  source 1..10: mol_type = other DNA
aagctagctt

SEQ ID NO: 33 - skipped

SEQ ID NO: 34 - DNA, 10 bp, synthetic construct
  misc_feature 1..10: note = Description of Artificial Sequence: Synthetic oligonucleotide
  source 1..10: mol_type = other DNA
aagctaagct